European Patent Specification EP 3 368 073 B1, published May 15, 2024. Title: A METHOD OF INHIBITING EXACERBATIONS OF T CELL-MEDIATED ALLOGRAFT VASCULOPATHY. Applicant: ALEXION PHARMACEUTICALS, INC. YALE UNIVERSITY. The sequence listing filed with the application follows.

SEQUENCE LISTING (36 sequences)

SEQ ID NO: 1 - protein, 10 aa, Artificial Sequence
  source: /note="Description of Artificial Sequence: Synthetic peptide"
GYIFSNYWIQ

SEQ ID NO: 2 - protein, 17 aa, Artificial Sequence
  source: /note="Description of Artificial Sequence: Synthetic peptide"
EILPGSGSTEYTENFKD

SEQ ID NO: 3 - protein, 13 aa, Artificial Sequence
  source: /note="Description of Artificial Sequence: Synthetic peptide"
YFFGSSPNWYFDV

SEQ ID NO: 4 - protein, 11 aa, Artificial Sequence
  source: /note="Description of Artificial Sequence: Synthetic peptide"
GASENIYGALN

SEQ ID NO: 5 - protein, 7 aa, Artificial Sequence
  source: /note="Description of Artificial Sequence: Synthetic peptide"
GATNLAD

SEQ ID NO: 6 - protein, 9 aa, Artificial Sequence
  source: /note="Description of Artificial Sequence: Synthetic peptide"
QNVLNTPLT

SEQ ID NO: 7 - protein, 122 aa, Artificial Sequence [sequence omitted]

SEQ ID NO: 8 - protein, 107 aa, Artificial Sequence [sequence omitted]

SEQ ID NO: 9 - protein, 326 aa, Artificial Sequence
  source: /note="Description of Artificial Sequence: Synthetic polypeptide"
ASTKGPSVFPLAPCSRSTSESTAALGCLVKDYFPEPVTVSWNSGALTSGVHTFPAVLQSSGLYSLSSVVTVPSSNFGTQTYTCNVDHKPSNTKVDKTVERKCCVECPPCPAPPVAGPSVFLFPPKPKDTLMISRTPEVTCVVVDVSQEDPEVQFNWYVDGVEVHNAKTKPREEQFNSTYRVVSVLTVLHQDWLNGKEYKCKVSNKGLPSSIEKTISKAKGQPREPQVYTLPPSQEEMTKNQVSLTCLVKGFYPSDIAVEWESNGQPENNYKTTPPVLDSDGSFFLYSRLTVDKSRWQEGNVFSCSVMHEALHNHYTQKSLSLSLGK

SEQ ID NO: 10 - protein, 448 aa, Artificial Sequence
  source: /note="Description of Artificial Sequence: Synthetic polypeptide"
QVQLVQSGAEVKKPGASVKVSCKASGYIFSNYWIQWVRQAPGQGLEWMGEILPGSGSTEYTENFKDRVTMTRDTSTSTVYMELSSLRSEDTAVYYCARYFFGSSPNWYFDVWGQGTLVTVSSASTKGPSVFPLAPCSRSTSESTAALGCLVKDYFPEPVTVSWNSGALTSGVHTFPAVLQSSGLYSLSSVVTVPSSNFGTQTYTCNVDHKPSNTKVDKTVERKCCVECPPCPAPPVAGPSVFLFPPKPKDTLMISRTPEVTCVVVDVSQEDPEVQFNWYVDGVEVHNAKTKPREEQFNSTYRVVSVLTVLHQDWLNGKEYKCKVSNKGLPSSIEKTISKAKGQPREPQVYTLPPSQEEMTKNQVSLTCLVKGFYPSDIAVEWESNGQPENNYKTTPPVLDSDGSFFLYSRLTVDKSRWQEGNVFSCSVMHEALHNHYTQKSLSLSLGK

SEQ ID NO: 11 - protein, 214 aa, Artificial Sequence [sequence omitted]

SEQ ID NO: 12 - protein, 122 aa, Artificial Sequence [sequence omitted]

SEQ ID NO: 13 - protein, 326 aa, Artificial Sequence
  source: /note="Description of Artificial Sequence: Synthetic polypeptide"
ASTKGPSVFPLAPCSRSTSESTAALGCLVKDYFPEPVTVSWNSGALTSGVHTFPAVLQSSGLYSLSSVVTVPSSNFGTQTYTCNVDHKPSNTKVDKTVERKCCVECPPCPAPPVAGPSVFLFPPKPKDTLMISRTPEVTCVVVDVSQEDPEVQFNWYVDGVEVHNAKTKPREEQFNSTYRVVSVLTVLHQDWLNGKEYKCKVSNKGLPSSIEKTISKAKGQPREPQVYTLPPSQEEMTKNQVSLTCLVKGFYPSDIAVEWESNGQPENNYKTTPPVLDSDGSFFLYSRLTVDKSRWQEGNVFSCSVLHEALHSHYTQKSLSLSLGK

SEQ ID NO: 14 - protein, 448 aa, Artificial Sequence
  source: /note="Description of Artificial Sequence: Synthetic polypeptide"
QVQLVQSGAEVKKPGASVKVSCKASGHIFSNYWIQWVRQAPGQGLEWMGEILPGSGHTEYTENFKDRVTMTRDTSTSTVYMELSSLRSEDTAVYYCARYFFGSSPNWYFDVWGQGTLVTVSSASTKGPSVFPLAPCSRSTSESTAALGCLVKDYFPEPVTVSWNSGALTSGVHTFPAVLQSSGLYSLSSVVTVPSSNFGTQTYTCNVDHKPSNTKVDKTVERKCCVECPPCPAPPVAGPSVFLFPPKPKDTLMISRTPEVTCVVVDVSQEDPEVQFNWYVDGVEVHNAKTKPREEQFNSTYRVVSVLTVLHQDWLNGKEYKCKVSNKGLPSSIEKTISKAKGQPREPQVYTLPPSQEEMTKNQVSLTCLVKGFYPSDIAVEWESNGQPENNYKTTPPVLDSDGSFFLYSRLTVDKSRWQEGNVFSCSVLHEALHSHYTQKSLSLSLGK

SEQ ID NO: 15 - protein, 326 aa, Artificial Sequence
  source: /note="Description of Artificial Sequence: Synthetic polypeptide"
ASTKGPSVFPLAPCSRSTSESTAALGCLVKDYFPEPVTVSWNSGALTSGVHTFPAVLQSSGLYSLSSVVTVTSSNFGTQTYTCNVDHKPSNTKVDKTVERKCCVECPPCPAPPVAGPSVFLFPPKPKDTLYITREPEVTCVVVDVSHEDPEVQFNWYVDGMEVHNAKTKPREEQFNSTFRVVSVLTVVHQDWLNGKEYKCKVSNKGLPAPIEKTISKTKGQPREPQVYTLPPSREEMTKNQVSLTCLVKGFYPSDIAVEWESNGQPENNYKTTPPMLDSDGSFFLYSKLTVDKSRWQQGNVFSCSVMHEALHNHYTQKSLSLSPGK

SEQ ID NO: 16 - protein, 448 aa, Artificial Sequence
  source: /note="Description of Artificial Sequence: Synthetic polypeptide"
QVQLVQSGAEVKKPGASVKVSCKASGYIFSNYWIQWVRQAPGQGLEWMGEILPGSGSTEYTENFKDRVTMTRDTSTSTVYMELSSLRSEDTAVYYCARYFFGSSPNWYFDVWGQGTLVTVSSASTKGPSVFPLAPCSRSTSESTAALGCLVKDYFPEPVTVSWNSGALTSGVHTFPAVLQSSGLYSLSSVVTVTSSNFGTQTYTCNVDHKPSNTKVDKTVERKCCVECPPCPAPPVAGPSVFLFPPKPKDTLYITREPEVTCVVVDVSHEDPEVQFNWYVDGMEVHNAKTKPREEQFNSTFRVVSVLTVVHQDWLNGKEYKCKVSNKGLPAPIEKTISKTKGQPREPQVYTLPPSREEMTKNQVSLTCLVKGFYPSDIAVEWESNGQPENNYKTTPPMLDSDGSFFLYSKLTVDKSRWQQGNVFSCSVMHEALHNHYTQKSLSLSPGK

SEQ ID NO: 17 - protein, 11 aa, Artificial Sequence
  source: /note="Description of Artificial Sequence: Synthetic peptide"
GASENIYHALN

SEQ ID NO: 18 - protein, 17 aa, Artificial Sequence
  source: /note="Description of Artificial Sequence: Synthetic peptide"
EILPGSGHTEYTENFKD

SEQ ID NO: 19 - protein, 10 aa, Artificial Sequence
  source: /note="Description of Artificial Sequence: Synthetic peptide"
GHIFSNYWIQ

SEQ ID NO: 20 - protein, 448 aa, Artificial Sequence
  source: /note="Description of Artificial Sequence: Synthetic polypeptide"
QVQLVQSGAEVKKPGASVKVSCKASGHIFSNYWIQWVRQAPGQGLEWMGEILPGSGHTEYTENFKDRVTMTRDTSTSTVYMELSSLRSEDTAVYYCARYFFGSSPNWYFDVWGQGTLVTVSSASTKGPSVFPLAPCSRSTSESTAALGCLVKDYFPEPVTVSWNSGALTSGVHTFPAVLQSSGLYSLSSVVTVPSSNFGTQTYTCNVDHKPSNTKVDKTVERKCCVECPPCPAPPVAGPSVFLFPPKPKDTLMISRTPEVTCVVVDVSQEDPEVQFNWYVDGVEVHNAKTKPREEQFNSTYRVVSVLTVLHQDWLNGKEYKCKVSNKGLPSSIEKTISKAKGQPREPQVYTLPPSQEEMTKNQVSLTCLVKGFYPSDIAVEWESNGQPENNYKTTPPVLDSDGSFFLYSRLTVDKSRWQEGNVFSCSVMHEALHNHYTQKSLSLSLGK

SEQ ID NO: 21 - protein, 5 aa, Artificial Sequence
  source: /note="Description of Artificial Sequence: Synthetic peptide"
SYAIS

SEQ ID NO: 22 - protein, 17 aa, Artificial Sequence
  source: /note="Description of Artificial Sequence: Synthetic peptide"
GIGPFFGTANYAQKFQG

SEQ ID NO: 23 - protein, 7 aa, Artificial Sequence
  source: /note="Description of Artificial Sequence: Synthetic peptide"
DTPYFDY

SEQ ID NO: 24 - protein, 11 aa, Artificial Sequence
  source: /note="Description of Artificial Sequence: Synthetic peptide"
SGDSIPNYYVY

SEQ ID NO: 25 - protein, 7 aa, Artificial Sequence
  source: /note="Description of Artificial Sequence: Synthetic peptide"
DDSNRPS

SEQ ID NO: 26 - protein, 11 aa, Artificial Sequence
  source: /note="Description of Artificial Sequence: Synthetic peptide"
QSFDSSLNAEV

SEQ ID NO: 27 - protein, 116 aa, Artificial Sequence
  source: /note="Description of Artificial Sequence: Synthetic polypeptide"
QVQLVQSGAEVKKPGSSVKVSCKASGGTFSSYAISVWRQAPGQGLEWMGGIGPFFGTANYAQKFQGRVTITADESTSTAYMELSSLRSEDTAVYYCARDTPYFDYWGQGTLVTVSS

SEQ ID NO: 28 - protein, 108 aa, Artificial Sequence
  source: /note="Description of Artificial Sequence: Synthetic polypeptide"
DIELTQPPSVSVAPGQTARISCSGDSIPNYYVYWYQQKPGQAPVLVIYDDSNRPSGIPERFSGSNSGNTATLTISGTQAEDEADYYCQSFDSSLNAEVFGGGTKLTVL

SEQ ID NO: 29 - protein, 4 aa, Artificial Sequence
  source: /note="Description of Artificial Sequence: Synthetic peptide"
NYIS

SEQ ID NO: 30 - protein, 17 aa, Artificial Sequence
  source: /note="Description of Artificial Sequence: Synthetic peptide"
IIDPDDSYTEYSPSFQG

SEQ ID NO: 31 - protein, 8 aa, Artificial Sequence
  source: /note="Description of Artificial Sequence: Synthetic peptide"
YEYGGFDI

SEQ ID NO: 32 - protein, 11 aa, Artificial Sequence
  source: /note="Description of Artificial Sequence: Synthetic peptide"
SGDNIGNSYVH

SEQ ID NO: 33 - protein, 7 aa, Artificial Sequence
  source: /note="Description of Artificial Sequence: Synthetic peptide"
KDNDRPS

SEQ ID NO: 34 - protein, 9 aa, Artificial Sequence
  source: /note="Description of Artificial Sequence: Synthetic peptide"
GTYDIESYV

SEQ ID NO: 35 - protein, 116 aa, Artificial Sequence
  source: /note="Description of Artificial Sequence: Synthetic polypeptide"
EVQLVQSGAEVKKPGESLKISCKGSGYSFTNYISWVRQMPGKGLEWMGIIDPDDSYTEYSPSFQGQVTISADKSISTAYLQWSSLKASDTAMYYCARYEYGGFDIWGQGTLVTVSS

SEQ ID NO: 36 - protein, 106 aa, Artificial Sequence
  source: /note="Description of Artificial Sequence: Synthetic polypeptide"
SYELTQPPSVSVAPGQTARISCSGDNIGNSYVHWYQQKPGQAPVLVIYKDNDRPSGIPERFSGSNSGNTATLTISGTQAEDEADYYCGTYDIESYVFGGGTKLTVL